European Patent Specification EP 3 875 104 B1, published January 22, 2025. Title: COMPOSITIONS FOR TREATING MYELOFIBROSIS. Applicant: Acceleron Pharma Inc. The sequence listing filed with the application follows.

SEQUENCE LISTING (46 sequences)

SEQ ID NO: 1 - protein, 512 aa, Homo sapiens
MTAPWVALALLWGSLWPGSGRGEAETRECIYYNANWELERTNQSGLERCEGEQDKRLHCYASWRNSSGTIELVKKGCWLDDFNCYDRQECVATEENPQVYFCCCEGNFCNERFTHLPEAGGPEVTYEPPPTAPTLLTVLAYSLLPIGGLSLIVLLAFWMYRHRKPPYGHVDIHEDPGPPPPSPLVGLKPLQLLEIKARGRFGCVWKAQLMNDFVAVKIFPLQDKQSWQSEREIFSTPGMKHENLLQFIAAEKRGSNLEVELWLITAFHDKGSLTDYLKGNIITWNELCHVAETMSRGLSYLHEDVPWCRGEGHKPSIAHRDFKSKNVLLKSDLTAVLADFGLAVRFEPGKPPGDTHGQVGTRRYMAPEVLEGAINFQRDAFLRIDMYAMGLVLWELVSRCKAADGPVDEYMLPFEEEIGQHPSLEELQEVVVHKKMRPTIKDHWLKHPGLAQLCVTIEECWDHDAEARLSAGCVEERVSLIRRSVNGTTSDCLVSLVTSVTNVDLPPKESSI

SEQ ID NO: 2 - protein, 115 aa, Homo sapiens
GRGEAETRECIYYNANWELERTNQSGLERCEGEQDKRLHCYASWRNSSGTIELVKKGCWLDDFNCYDRQECVATEENPQVYFCCCEGNFCNERFTHLPEAGGPEVTYEPPPTAPT

SEQ ID NO: 3 - protein, 100 aa, Homo sapiens
GRGEAETRECIYYNANWELERTNQSGLERCEGEQDKRLHCYASWRNSSGTIELVKKGCWLDDFNCYDRQECVATEENPQVYFCCCEGNFCNERFTHLPEA

SEQ ID NO: 4 - DNA, 1539 bp, Homo sapiens
atgacggcgccctgggtggccctcgccctcctctggggatcgctgtggcccggctctgggcgtggggaggctgagacacgggagtgcatctactacaacgccaactgggagctggagcgcaccaaccagagcggcctggagcgctgcgaaggcgagcaggacaagcggctgcactgctacgcctcctgggccaacagctctggcaccatcgagctcgtgaagaagggctgctggctagatgacttcaactgctacgataggcaggagtgtgtggccactgaggagaacccccaggtgtacttctgctgctgtgaaggcaacttctgcaacgagcgcttcactcatttgccagaggctgggggcccggaagtcacgtacgagccacccccgacagcccccaccctgctcacggtgctggcctactcactgctgcccatcgggggcctttccctcatcgtcctgctggccttttggatgtaccggcatcgcaagcccccctacggtcatgtggacatccatgaggaccctgggcctccaccaccatcccctctggtgggcctgaagccactgcagctgctggagatcaaggctcgggggcgctttggctgtgtctggaaggcccagctcatgaatgactttgtagctgtcaagatcttcccactccaggacaagcagtcgtggcagagtgaacgggagatcttcagcacacctggcatgaagcacgagaacctgctacagttcattgctgccgagaagcgaggctccaacctcgaagtagagctgtggctcatcacggccttccatgacaagggctccctcacggattacctcaaggggaacatcatcacatggaacgaactgtgtcatgtagcagagacgatgtcacgaggcctctcatacctgcatgaggatgtgccctggtgccgtggcgagggccacaagccgtctattgcccacagggactttaaaagtaagaatgtattgctgaagagcgacctcacagccgtgctggctgactttggcttggctgttcgatttgagccagggaaacctccaggggacacccacggacaggtaggcacgagacggtacatggctcctgaggtgctcgagggagccatcaacttccagagagatgccttcctgcgcattgacatgtatgccatggggttggtgctgtgggagcttgtgtctcgctgcaaggctgcagacggacccgtggatgagtacatgctgccctttgaggaagagattggccagcacccttcgttggaggagctgcaggaggtggtggtgcacaagaagatgaggcccaccattaaagatcactggttgaaacacccgggcctggcccagctttgtgtgaccatcgaggagtgctgggaccatgatgcagaggctcgcttgtccgcgggctgtgtggaggagcgggtgtccctgattcggaggtcggtcaacggcactacctcggactgtctcgtttccctggtgacctctgtcaccaatgtggacctgccccctaaagagtcaagcatctaa

SEQ ID NO: 5 - DNA, 345 bp, Homo sapiens
gggcgtggggaggctgagacacgggagtgcatctactacaacgccaactgggagctggagcgcaccaaccagagcggcctggagcgctgcgaaggcgagcaggacaagcggctgcactgctacgcctcctgggccaacagctctggcaccatcgagctcgtgaagaagggctgctggctagatgacttcaactgctacgataggcaggagtgtgtggccactgaggagaacccccaggtgtacttctgctgctgtgaaggcaacttctgcaacgagcgcttcactcatttgccagaggctgggggcccggaagtcacgtacgagccacccccgacagcccccacc

SEQ ID NO: 6 - protein, 225 aa, Artificial Sequence
  Description of Artificial Sequence: Synthetic polypeptide
  MOD_RES (43)..(43): Asp or Ala
  MOD_RES (100)..(100): Lys or Ala
  MOD_RES (212)..(212): Asn or Ala
THTCPPCPAPELLGGPSVFLFPPKPKDTLMISRTPEVTCVVVXVSHEDPEVKFNWYVDGVEVHNAKTKPREEQYNSTYRVVSVLTVLHQDWLNGKEYKCXVSNKALPVPIEKTISKAKGQPREPQVYTLPPSREEMTKNQVSLTCLVKGFYPSDIAVEWESNGQPENNYKTTPPVLDSDGPFFLYSKLTVDKSRWQQGNVFSCSVMHEALHXHYTQKSLSLSPGK

SEQ ID NO: 7 - protein, 343 aa, Artificial Sequence
  Description of Artificial Sequence: Synthetic polypeptide
GRGEAETRECIYYNANWELERTNQSGLERCEGEQDKRLHCYASWRNSSGTIELVKKGCWDDDFNCYDRQECVATEENPQVYFCCCEGNFCNERFTHLPEAGGPEVTYEPPPTAPTGGGTHTCPPCPAPELLGGPSVFLFPPKPKDTLMISRTPEVTCVVVDVSHEDPEVKFNWYVDGVEVHNAKTKPREEQYNSTYRVVSVLTVLHQDWLNGKEYKCKVSNKALPVPIEKTISKAKGQPREPQVYTLPPSREEMTKNQVSLTCLVKGFYPSDIAVEWESNGQPENNYKTTPPVLDSDGSFFLYSKLTVDKSRWQQGNVFSCSVMHEALHNHYTQKSLSLSPGK

SEQ ID NO: 8 - protein, 21 aa, Unknown
  Description of Unknown: Honey bee mellitin peptide
MKFLVNVALVFMVVYISYIYA

SEQ ID NO: 9 - protein, 22 aa, Unknown
  Description of Unknown: Tissue plasminogen activator peptide
MDAMKRGLCCVLLLCGAVFVSP

SEQ ID NO: 10 - protein, 19 aa, Unknown
  Description of Unknown: Native leader peptide
MTAPWVALALLWGSLCAGS

SEQ ID NO: 11 - protein, 368 aa, Artificial Sequence
  Description of Artificial Sequence: Synthetic polypeptide
MDAMKRGLCCVLLLCGAVFVSPGASGRGEAETRECIYYNANWELERTNQSGLERCEGEQDKRLHCYASWRNSSGTIELVKKGCWDDDFNCYDRQECVATEENPQVYFCCCEGNFCNERFTHLPEAGGPEVTYEPPPTAPTGGGTHTCPPCPAPELLGGPSVFLFPPKPKDTLMISRTPEVTCVVVDVSHEDPEVKFNWYVDGVEVHNAKTKPREEQYNSTYRVVSVLTVLHQDWLNGKEYKCKVSNKALPVPIEKTISKAKGQPREPQVYTLPPSREEMTKNQVSLTCLVKGFYPSDIAVEWESNGQPENNYKTTPPVLDSDGSFFLYSKLTVDKSRWQQGNVFSCSVMHEALHNHYTQKSLSLSPGK

SEQ ID NO: 12 - DNA, 1107 bp, Artificial Sequence
  Description of Artificial Sequence: Synthetic polynucleotide
atggatgcaatgaagagagggctctgctgtgtgctgctgctgtgtggagcagtcttcgtttcgcccggcgcctctgggcgtggggaggctgagacacgggagtgcatctactacaacgccaactgggagctggagcgcaccaaccagagcggcctggagcgctgcgaaggcgagcaggacaagcggctgcactgctacgcctcctggcgcaacagctctggcaccatcgagctcgtgaagaagggctgctgggacgatgacttcaactgctacgataggcaggagtgtgtggccactgaggagaacccccaggtgtacttctgctgctgtgaaggcaacttctgcaacgagcgcttcactcatttgccagaggctgggggcccggaagtcacgtacgagccacccccgacagcccccaccggtggtggaactcacacatgcccaccgtgcccagcacctgaactcctggggggaccgtcagtcttcctcttccccccaaaacccaaggacaccctcatgatctcccggacccctgaggtcacatgcgtggtggtggacgtgagccacgaagaccctgaggtcaagttcaactggtacgtggacggcgtggaggtgcataatgccaagacaaagccgcgggaggagcagtacaacagcacgtaccgtgtggtcagcgtcctcaccgtcctgcaccaggactggctgaatggcaaggagtacaagtgcaaggtctccaacaaagccctcccagtccccatcgagaaaaccatctccaaagccaaagggcagccccgagaaccacaggtgtacaccctgcccccatcccgggaggagatgaccaagaaccaggtcagcctgacctgcctggtcaaaggcttctatcccagcgacatcgccgtggagtgggagagcaatgggcagccggagaacaactacaagaccacgcctcccgtgctggactccgacggctccttcttcctctatagcaagctcaccgtggacaagagcaggtggcagcaggggaacgtcttctcatgctccgtgatgcatgaggctctgcacaaccactacacgcagaagagcctctccctgtctccgggtaaatga

SEQ ID NO: 13 - protein, 5 aa, Artificial Sequence
  Description of Artificial Sequence: Synthetic peptide
TGGGG

SEQ ID NO: 14 - protein, 5 aa, Artificial Sequence
  Description of Artificial Sequence: Synthetic peptide
SGGGG

SEQ ID NO: 15 - protein, 116 aa, Homo sapiens
ILGRSETQECLFFNANWEKDRTNQTGVEPCYGDKDKRRHCFATWKNISGSIEIVKQGCWLDDINCYDRTDCVEKKDSPEVYFCCCEGNMCNEKFSYFPEMEVTQPTSNPVTPKPPT

SEQ ID NO: 16 - protein, 150 aa, Rattus sp.
MTAPWAALALLWGSLCAGSGRGEAETRECIYYNANWELERTNQSGLERCEGEQDKRLHCYASWPNSSGTIELVKKGCWLDDFNCYDRQECVATEENPQVYFCCCEGNFCNERFTHLPEPGGPEVTYEPPPTAPTLLTVLAYSLLPIGGLS

SEQ ID NO: 17 - protein, 150 aa, Sus sp.
MTAPWAALALLWGSLCVGSGRGEAETRECIYYNANWELERTNQSGLERCEGEQDKRLHCYASWRNSSGTIELVKKGCWLDDFNCYDRQECVATEENPQVYFCCCEGNFCNERFTHLPEAGGPEVTYEPPPTAPTLLTVLAYSLLPIGGLS

SEQ ID NO: 18 - protein, 150 aa, Mus sp.
MTAPWAALALLWGSLCAGSGRGEAETRECIYYNANWELERTNQSGLERCEGEQDKRLHCYASWRNSSGTIELVKKGCWLDDFNCYDRQECVATEENPQVYFCCCEGNFCNERFTHLPEPGGPEVTYEPPPTAPTLLTVLAYSLLPIGGLS

SEQ ID NO: 19 - protein, 150 aa, Homo sapiens
MTAPWVALALLWGSLCAGSGRGEAETRECIYYNANWELERTNQSGLERCEGEQDKRLHCYASWRNSSGTIELVKKGCWLDDFNCYDRQECVATEENPQVYFCCCEGNFCNERFTHLPEAGGPEVTYEPPPTAPTLLTVLAYSLLPIGGLS

SEQ ID NO: 20 - protein, 150 aa, Bos sp.
MTAPWAALALLWGSLCAGSGRGEAETRECIYYNANWELERTNQSGLERCEGERDKRLHCYASWRNSSGTIELVKKGCWLDDFNCYDRQECVATEENPQVYFCCCEGNFCNERFTHLPEAGGPEVTYEPPPTAPTLLTVLAYSLLPVGGLS

SEQ ID NO: 21 - protein, 150 aa, Xenopus sp.
MGASVALTFLLLLATFRAGSGHDEVETRECIYYNANWELEKTNQSGVERLVEGKKDKRLHCYASWRNNSGFIELVKKGCWLDDFNCYDRQECIAKEENPQVFFCCCEGNYCNKKFTHLPEVETFDPKPQPSASVLNILIYSLLPIVGLSM

SEQ ID NO: 22 - protein, 150 aa, Homo sapiens
MGAAAKLAFAVFLISCSSGAILGRSETQECLFFNANWEKDRTNQTGVEPCYGDKDKRRHCFATWKNISGSIEIVKQGCWLDDINCYDRTDCVEKKDSPEVYFCCCEGNMCNEKFSYFPEMEVTQPTSNPVTPKPPYYNILLYSLVPLMLI

SEQ ID NO: 23 - protein, 154 aa, Artificial Sequence
  Description of Artificial Sequence: Synthetic consensus polypeptide
  MOD_RES (8)..(8): Thr, Ala or not present
  MOD_RES (121)..(121): Pro, Ala, Val or Met
MTAPWAAXLALLWGSLCAGSGRGEAETRECIYYNANWELERTNQSGLERLCEGEQDKRLHCYASWRNSSGTIELVKKGCWLDDFNCYDRQECVATEENPQVYFCCCEGNFCNERFTHLPEXGGPEVTYEPKPPTAPTLLTVLAYSLLPIGGLSM

SEQ ID NO: 24 - protein, 6 aa, Artificial Sequence
  Description of Artificial Sequence: Synthetic 6xHis tag
HHHHHH

SEQ ID NO: 25 - DNA, 1107 bp, Artificial Sequence
  Description of Artificial Sequence: Synthetic polynucleotide
atggatgcaatgaagagagggctctgctgtgtgctgctgctgtgtggagcagtcttcgtttcgcccggcgcctctgggcgtggggaggctgagacacgggagtgcatctactacaacgccaactgggagctggagcgcaccaaccagagcggcctggagcgctgcgaaggcgagcaggacaagcggctgcactgctacgcctcctggcgcaacagctctggcaccatcgagctcgtgaagaagggctgctgggatgatgacttcaactgctacgataggcaggagtgtgtggccactgaggagaacccccaggtgtacttctgctgctgtgaaggcaacttctgcaacgagcgcttcactcatttgccagaggctgggggcccggaagtcacgtacgagccacccccgacagcccccaccggtggtggaactcacacatgcccaccgtgcccagcacctgaactcctggggggaccgtcagtcttcctcttccccccaaaacccaaggacaccctcatgatctcccggacccctgaggtcacatgcgtggtggtggacgtgagccacgaagaccctgaggtcaagttcaactggtacgtggacggcgtggaggtgcataatgccaagacaaagccgcgggaggagcagtacaacagcacgtaccgtgtggtcagcgtcctcaccgtcctgcaccaggactggctgaatggcaaggagtacaagtgcaaggtctccaacaaagccctcccagcccccatcgagaaaaccatctccaaagccaaagggcagccccgagaaccacaggtgtacaccctgcccccatcccgggaggagatgaccaagaaccaggtcagcctgacctgcctggtcaaaggcttctatcccagcgacatcgccgtggagtgggagagcaatgggcagccggagaacaactacaagaccacgcctcccgtgctggactccgacggctccttcttcctctatagcaagctcaccgtggacaagagcaggtggcagcaggggaacgtcttctcatgctccgtgatgcatgaggctctgcacaaccactacacgcagaagagcctctccctgtccccgggtaaatga

SEQ ID NO: 26 - protein, 360 aa, Artificial Sequence
  Description of Artificial Sequence: Synthetic polypeptide
MDAMKRGLCCVLLLCGAVFVSPGAAETRECIYYNANWELERTNQSGLERCEGEQDKRLHCYASWRNSSGTIELVKKGCWDDDFNCYDRQECVATEENPQVYFCCCEGNFCNERFTHLPEAGGPEVTYEPPPTGGGTHTCPPCPAPELLGGPSVFLFPPKPKDTLMISRTPEVTCVVVDVSHEDPEVKFNWYVDGVEVHNAKTKPREEQYNSTYRVVSVLTVLHQDWLNGKEYKCKVSNKALPAPIEKTISKAKGQPREPQVYTLPPSREEMTKNQVSLTCLVKGFYPSDIAVEWESNGQPENNYKTTPPVLDSDGSFFLYSKLTVDKSRWQQGNVFSCSVMHEALHNHYTQKSLSLSPGK

SEQ ID NO: 27 - DNA, 1083 bp, Artificial Sequence
  Description of Artificial Sequence: Synthetic polynucleotide
  CDS (76)..(396)
atggatgcaatgaagagagggctctgctgtgtgctgctgctgtgtggagcagtcttcgtttcgcccggcgccgctgagacacgggagtgcatctactacaacgccaactgggagctggagcgcaccaaccagagcggcctggagcgctgcgaaggcgagcaggacaagcggctgcactgctacgcctcctggcgcaacagctctggcaccatcgagctcgtgaagaagggctgctgggacgatgacttcaactgctacgataggcaggagtgtgtggccactgaggagaacccccaggtgtacttctgctgctgtgaaggcaacttctgcaacgagcgcttcactcatttgccagaggctgggggcccggaagtcacgtacgagccacccccgacaggtggtggaactcacacatgcccaccgtgcccagcacctgaactcctggggggaccgtcagtcttcctcttccccccaaaacccaaggacaccctcatgatctcccggacccctgaggtcacatgcgtggtggtggacgtgagccacgaagaccctgaggtcaagttcaactggtacgtggacggcgtggaggtgcataatgccaagacaaagccgcgggaggagcagtacaacagcacgtaccgtgtggtcagcgtcctcaccgtcctgcaccaggactggctgaatggcaaggagtacaagtgcaaggtctccaacaaagccctcccagcccccatcgagaaaaccatctccaaagccaaagggcagccccgagaaccacaggtgtacaccctgcccccatcccgggaggagatgaccaagaaccaggtcagcctgacctgcctggtcaaaggcttctatcccagcgacatcgccgtggagtgggagagcaatgggcagccggagaacaactacaagaccacgcctcccgtgctggactccgacggctccttcttcctctatagcaagctcaccgtggacaagagcaggtggcagcaggggaacgtcttctcatgctccgtgatgcatgaggctctgcacaaccactacacgcagaagagcctctccctgtccccgggtaaatga

SEQ ID NO: 28 - protein, 335 aa, Artificial Sequence
  Description of Artificial Sequence: Synthetic polypeptide
ETRECIYYNANWELERTNQSGLERCEGEQDKRLHCYASWRNSSGTIELVKKGCWDDDFNCYDRQECVATEENPQVYFCCCEGNFCNERFTHLPEAGGPEVTYEPPPTGGGTHTCPPCPAPELLGGPSVFLFPPKPKDTLMISRTPEVTCVVVDVSHEDPEVKFNWYVDGVEVHNAKTKPREEQYNSTYRVVSVLTVLHQDWLNGKEYKCKVSNKALPAPIEKTISKAKGQPREPQVYTLPPSREEMTKNQVSLTCLVKGFYPSDIAVEWESNGQPENNYKTTPPVLDSDGSFFLYSKLTVDKSRWQQGNVFSCSVMHEALHNHYTQKSLSLSPGK

SEQ ID NO: 29 - protein, 107 aa, Artificial Sequence
  Description of Artificial Sequence: Synthetic polypeptide
ETRECIYYNANWELERTNQSGLERCEGEQDKRLHCYASWRNSSGTIELVKKGCWDDDFNCYDRQECVATEENPQVYFCCCEGNFCNERFTHLPEAGGPEVTYEPPPT

SEQ ID NO: 30 - DNA, 1083 bp, Artificial Sequence
  Description of Artificial Sequence: Synthetic polynucleotide
  CDS (76)..(396)
atggatgcaatgaagagagggctctgctgtgtgctgctgctgtgtggagcagtcttcgtttcgcccggcgccgccgaaacccgcgaatgtatttattacaatgctaattgggaactcgaacggacgaaccaatccgggctcgaacggtgtgagggggaacaggataaacgcctccattgctatgcgtcgtggaggaactcctccgggacgattgaactggtcaagaaagggtgctgggacgacgatttcaattgttatgaccgccaggaatgtgtcgcgaccgaagagaatccgcaggtctatttctgttgttgcgaggggaatttctgtaatgaacggtttacccacctccccgaagccggcgggcccgaggtgacctatgaacccccgcccaccggtggtggaactcacacatgcccaccgtgcccagcacctgaactcctggggggaccgtcagtcttcctcttccccccaaaacccaaggacaccctcatgatctcccggacccctgaggtcacatgcgtggtggtggacgtgagccacgaagaccctgaggtcaagttcaactggtacgtggacggcgtggaggtgcataatgccaagacaaagccgcgggaggagcagtacaacagcacgtaccgtgtggtcagcgtcctcaccgtcctgcaccaggactggctgaatggcaaggagtacaagtgcaaggtctccaacaaagccctcccagcccccatcgagaaaaccatctccaaagccaaagggcagccccgagaaccacaggtgtacaccctgcccccatcccgggaggagatgaccaagaaccaggtcagcctgacctgcctggtcaaaggcttctatcccagcgacatcgccgtggagtgggagagcaatgggcagccggagaacaactacaagaccacgcctcccgtgctggactccgacggctccttcttcctctatagcaagctcaccgtggacaagagcaggtggcagcaggggaacgtcttctcatgctccgtgatgcatgaggctctgcacaaccactacacgcagaagagcctctccctgtccccgggtaaatga

SEQ ID NO: 31 - DNA, 321 bp, Artificial Sequence
  Description of Artificial Sequence: Synthetic polynucleotide
gaaacccgcgaatgtatttattacaatgctaattgggaactcgaacggacgaaccaatccgggctcgaacggtgtgagggggaacaggataaacgcctccattgctatgcgtcgtggaggaactcctccgggacgattgaactggtcaagaaagggtgctgggacgacgatttcaattgttatgaccgccaggaatgtgtcgcgaccgaagagaatccgcaggtctatttctgttgttgcgaggggaatttctgtaatgaacggtttacccacctccccgaagccggcgggcccgaggtgacctatgaacccccgcccacc

SEQ ID NO: 32 - protein, 115 aa, Artificial Sequence
  Description of Artificial Sequence: Synthetic polypeptide
GRGEAETRECIYYNANWELERTNQSGLERCEGEQDKRLHCYASWRNSSGTIELVKKGCWDDDFNCYDRQECVATEENPQVYFCCCEGNFCNERFTHLPEAGGPEVTYEPPPTAPT

SEQ ID NO: 33 - DNA, 1107 bp, Artificial Sequence
  Description of Artificial Sequence: Synthetic polynucleotide
tcatttacccggggacagggagaggctcttctgcgtgtagtggttgtgcagagcctcatgcatcacggagcatgagaagacgttcccctgctgccacctgctcttgtccacggtgagcttgctatagaggaagaaggagccgtcggagtccagcacgggaggcgtggtcttgtagttgttctccggctgcccattgctctcccactccacggcgatgtcgctgggatagaagcctttgaccaggcaggtcaggctgacctggttcttggtcatctcctcccgggatgggggcagggtgtacacctgtggttctcggggctgccctttggctttggagatggttttctcgatgggggctgggagggctttgttggagaccttgcacttgtactccttgccattcagccagtcctggtgcaggacggtgaggacgctgaccacacggtacgtgctgttgtactgctcctcccgcggctttgtcttggcattatgcacctccacgccgtccacgtaccagttgaacttgacctcagggtcttcgtggctcacgtccaccaccacgcatgtgacctcaggggtccgggagatcatgagggtgtccttgggttttggggggaagaggaagactgacggtccccccaggagttcaggtgctgggcacggtgggcatgtgtgagttccaccaccggtgggggctgtcgggggtggctcgtacgtgacttccgggcccccagcctctggcaaatgagtgaagcgctcgttgcagaagttgccttcacagcagcagaagtacacctgggggttctcctcagtggccacacactcctgcctatcgtagcagttgaagtcatcatcccagcagcccttcttcacgagctcgatggtgccagagctgttgcgccaggaggcgtagcagtgcagccgcttgtcctgctcgccttcgcagcgctccaggccgctctggttggtgcgctccagctcccagttggcgttgtagtagatgcactcccgtgtctcagcctccccacgcccagaggcgccgggcgaaacgaagactgctccacacagcagcagcacacagcagagccctctcttcattgcatccat

SEQ ID NO: 34 - DNA, 1083 bp, Artificial Sequence
  Description of Artificial Sequence: Synthetic polynucleotide
tcatttacccggggacagggagaggctcttctgcgtgtagtggttgtgcagagcctcatgcatcacggagcatgagaagacgttcccctgctgccacctgctcttgtccacggtgagcttgctatagaggaagaaggagccgtcggagtccagcacgggaggcgtggtcttgtagttgttctccggctgcccattgctctcccactccacggcgatgtcgctgggatagaagcctttgaccaggcaggtcaggctgacctggttcttggtcatctcctcccgggatgggggcagggtgtacacctgtggttctcggggctgccctttggctttggagatggttttctcgatgggggctgggagggctttgttggagaccttgcacttgtactccttgccattcagccagtcctggtgcaggacggtgaggacgctgaccacacggtacgtgctgttgtactgctcctcccgcggctttgtcttggcattatgcacctccacgccgtccacgtaccagttgaacttgacctcagggtcttcgtggctcacgtccaccaccacgcatgtgacctcaggggtccgggagatcatgagggtgtccttgggttttggggggaagaggaagactgacggtccccccaggagttcaggtgctgggcacggtgggcatgtgtgagttccaccacctgtcgggggtggctcgtacgtgacttccgggcccccagcctctggcaaatgagtgaagcgctcgttgcagaagttgccttcacagcagcagaagtacacctgggggttctcctcagtggccacacactcctgcctatcgtagcagttgaagtcatcgtcccagcagcccttcttcacgagctcgatggtgccagagctgttgcgccaggaggcgtagcagtgcagccgcttgtcctgctcgccttcgcagcgctccaggccgctctggttggtgcgctccagctcccagttggcgttgtagtagatgcactcccgtgtctcagcggcgccgggcgaaacgaagactgctccacacagcagcagcacacagcagagccctctcttcattgcatccat

SEQ ID NO: 35 - DNA, 1083 bp, Artificial Sequence
  Description of Artificial Sequence: Synthetic polynucleotide
tcatttacccggggacagggagaggctcttctgcgtgtagtggttgtgcagagcctcatgcatcacggagcatgagaagacgttcccctgctgccacctgctcttgtccacggtgagcttgctatagaggaagaaggagccgtcggagtccagcacgggaggcgtggtcttgtagttgttctccggctgcccattgctctcccactccacggcgatgtcgctgggatagaagcctttgaccaggcaggtcaggctgacctggttcttggtcatctcctcccgggatgggggcagggtgtacacctgtggttctcggggctgccctttggctttggagatggttttctcgatgggggctgggagggctttgttggagaccttgcacttgtactccttgccattcagccagtcctggtgcaggacggtgaggacgctgaccacacggtacgtgctgttgtactgctcctcccgcggctttgtcttggcattatgcacctccacgccgtccacgtaccagttgaacttgacctcagggtcttcgtggctcacgtccaccaccacgcatgtgacctcaggggtccgggagatcatgagggtgtccttgggttttggggggaagaggaagactgacggtccccccaggagttcaggtgctgggcacggtgggcatgtgtgagttccaccaccggtgggcgggggttcataggtcacctcgggcccgccggcttcggggaggtgggtaaaccgttcattacagaaattcccctcgcaacaacagaaatagacctgcggattctcttcggtcgcgacacattcctggcggtcataacaattgaaatcgtcgtcccagcaccctttcttgaccagttcaatcgtcccggaggagttcctccacgacgcatagcaatggaggcgtttatcctgttccccctcacaccgttcgagcccggattggttcgtccgttcgagttcccaattagcattgtaataaatacattcgcgggtttcggcggcgccgggcgaaacgaagactgctccacacagcagcagcacacagcagagccctctcttcattgcatccat

SEQ ID NO: 36 - protein, 141 aa, Homo sapiens
GRGEAETRECIYYNANWELERTNQSGLERCEGEQDKRLHCYASWRNSSGTIELVKKGCWLDDFNCYDRQECVATEENPQVYFCCCEGNFCNERFTHLPEAGGPEGPWASTTIPSGGPEATAAAGDQGSGALWLCLEGPAHE

SEQ ID NO: 37 - protein, 141 aa, Homo sapiens
GRGEAETRECIYYNANWELERTNQSGLERCEGEQDKRLHCYASWRNSSGTIELVKKGCWDDDFNCYDRQECVATEENPQVYFCCCEGNFCNERFTHLPEAGGPEGPWASTTIPSGGPEATAAAGDQGSGALWLCLEGPAHE

SEQ ID NO: 38 - protein, 370 aa, Artificial Sequence
  Description of Artificial Sequence: Synthetic polypeptide
GRGEAETRECIYYNANWELERTNQSGLERCEGEQDKRLHCYASWRNSSGTIELVKKGCWDDDFNCYDRQECVATEENPQVYFCCCEGNFCNERFTHLPEAGGPEGPWASTTIPSGGPEATAAAGDQGSGALWLCLEGPAHETGGGTHTCPPCPAPELLGGPSVFLFPPKPKDTLMISRTPEVTCVVVDVSHEDPEVKFNWYVDGVEVHNAKTKPREEQYNSTYRVVSVLTVLHQDWLNGKEYKCKVSNKALPAPIEKTISKAKGQPREPQVYTLPPSREEMTKNQVSLTCLVKGFYPSDIAVEWESNGQPENNYKTTPPVLDSDGSFFLYSKLTVDKSRWQQGNVFSCSVMHEALHNHYTQKSLSLSPGK

SEQ ID NO: 39 - protein, 512 aa, Homo sapiens
MTAPWVALALLWGSLWPGSGRGEAETRECIYYNANWELERTNQSGLERCEGEQDKRLHCYASWANSSGTIELVKKGCWLDDFNCYDRQECVATEENPQVYFCCCEGNFCNERFTHLPEAGGPEVTYEPPPTAPTLLTVLAYSLLPIGGLSLIVLLAFWMYRHRKPPYGHVDIHEDPGPPPPSPLVGLKPLQLLEIKARGRFGCVWKAQLMNDFVAVKIFPLQDKQSWQSEREIFSTPGMKHENLLQFIAAEKRGSNLEVELWLITAFHDKGSLTDYLKGNIITWNELCHVAETMSRGLSYLHEDVPWCRGEGHKPSIAHRDFKSKNVLLKSDLTAVLADFGLAVRFEPGKPPGDTHGQVGTRRYMAPEVLEGAINFQRDAFLRIDMYAMGLVLWELVSRCKAADGPVDEYMLPFEEEIGQHPSLEELQEVVVHKKMRPTIKDHWLKHPGLAQLCVTIEECWDHDAEARLSAGCVEERVSLIRRSVNGTTSDCLVSLVTSVTNVDLPPKESSI

SEQ ID NO: 40 - protein, 115 aa, Homo sapiens
GRGEAETRECIYYNANWELERTNQSGLERCEGEQDKRLHCYASWANSSGTIELVKKGCWLDDFNCYDRQECVATEENPQVYFCCCEGNFCNERFTHLPEAGGPEVTYEPPPTAPT

SEQ ID NO: 41 - protein, 100 aa, Homo sapiens
GRGEAETRECIYYNANWELERTNQSGLERCEGEQDKRLHCYASWANSSGTIELVKKGCWLDDFNCYDRQECVATEENPQVYFCCCEGNFCNERFTHLPEA

SEQ ID NO: 42 - protein, 10 aa, Artificial Sequence
  Description of Artificial Sequence: Synthetic peptide
  misc_feature (1)..(10): This sequence may encompass 2 to 10 residues
GGGGGGGGGG

SEQ ID NO: 43 - protein, 5 aa, Artificial Sequence
  Description of Artificial Sequence: Synthetic peptide
  misc_feature (1)..(5): This sequence may encompass 2 to 5 residues
GGGGG

SEQ ID NO: 44 - protein, 4 aa, Artificial Sequence
  Description of Artificial Sequence: Synthetic peptide
  misc_feature (1)..(4): This sequence may encompass 2 to 4 residues
GGGG

SEQ ID NO: 45 - protein, 4 aa, Artificial Sequence
  Description of Artificial Sequence: Synthetic peptide
TGGG

SEQ ID NO: 46 - protein, 368 aa, Artificial Sequence
  Description of Artificial Sequence: Synthetic polypeptide
MDAMKRGLCCVLLLCGAVFVSPGASGRGEAETRECIYYNANWELERTNQSGLERCEGEQDKRLHCYASWRNSSGTIELVKKGCWDDDFNCYDRQECVATEENPQVYFCCCEGNFCNERFTHLPEAGGPEVTYEPPPTAPTGGGTHTCPPCPAPELLGGPSVFLFPPKPKDTLMISRTPEVTCVVVDVSHEDPEVKFNWYVDGVEVHNAKTKPREEQYNSTYRVVSVLTVLHQDWLNGKEYKCKVSNKALPAPIEKTISKAKGQPREPQVYTLPPSREEMTKNQVSLTCLVKGFYPSDIAVEWESNGQPENNYKTTPPVLDSDGSFFLYSKLTVDKSRWQQGNVFSCSVMHEALHNHYTQKSLSLSPGK